European Patent Application EP 4 748 923 A1, published May 27, 2026. Title: 利用重组大肠杆菌生产L-精氨酸的方法及其所用重组菌. Applicant: 宁夏伊品生物科技股份有限公司. The sequence listing filed with the application follows.

SEQUENCE LISTING (51 sequences)

SEQ ID NO: 1 - DNA, 74 bp, synthetic construct
  source 1..74: mol_type = other DNA
ttgacaattaatcatccggctcgtataatgtgtggaattgtgagcggataacaatttcacacaggaaacagacc

SEQ ID NO: 2 - DNA, 1155 bp, Escherichia coli
  source 1..1155: mol_type = genomic DNA
atgctgctggtactggtgctgattggtcttaatatgcgaccactgctcacctccgtcgggccactgctaccgcaattgcgccaggcgagcggaatgagctttagcgtggctgccctgttgaccgctctgccggtggttaccatgggcgggctggcgctggccggaagctggcttcatcagcatgtcagcgaacgtcgcagtgtcgccatcagtctgttgctgattgccgtcggtgcattgatgcgtgagctttacccgcaaagtgcgctgctgcttagcagcgcactgcttggtggggtggggatcggcatcattcaggcggtgatgccttcggtgattaaacggcggtttcagcagcgcacgccactggtgatggggctgtggtccgcggctctgatgggcggcggtgggcttggtgccgccataacgccctggttagttcaacatagcgaaacctggtatcaaacactcgcctggtgggcgctgcctgccgttgttgcgctctttgcctggtggtggcaaagcgcccgcgaggtcgcctcttcccacaagacaacaaccactccggttcgcgtggtattcactccccgcgcgtggacgctgggtgtttacttcggtctgattaacggcggttacgccagcctgattgcctggttacccgctttctatattgagattggtgccagcgcgcagtacagcggttccttactggcattgatgacgcttgggcaagccgcaggagctttgctgatgcctgctatggctcgccatcaggatcggcgcaaactgttaatgctggcgctggtgttacaactggtggggttctgcggctttatctggctgccgatgcaattgccggtattgtgggcgatggtgtgtgggttaggtctgggcggcgcgtttccgctctgtttgctgctggcgctcgatcactctgtgcaaccggctattgctggcaagctggtggcgtttatgcagggaatcggttttatcatcgccgggcttgccccgtggttttctggcgtgctgcgtagtatcagcggcaattacctgatggactgggcatttcatgcgctgtgcgtcgttgggctgatgatcataaccctgcgttttgcaccagtacgttttccgcagctgtgggtcaaagaggcatga

SEQ ID NO: 3 - DNA, 660 bp, Escherichia coli
  source 1..660: mol_type = genomic DNA
gtgaaagagattattgatggattccttaaattccagcgcgaggcatttccgaagcgggaagccttgtttaaacagctggcgacacagcaaagcccgcgcacactttttatctcctgctccgacagccgtctggtccctgagctggtgacgcaacgtgagcctggcgatctgttcgttattcgcaacgcgggcaatatcgtcccttcctacgggccggaacccggtggcgtttctgcttcggtggagtatgccgtcgctgcgcttcgggtatctgacattgtgatttgtggtcattccaactgtggcgcgatgaccgccattgccagctgtcagtgcatggaccatatgcctgccgtctcccactggctgcgttatgccgattcagcccgcgtcgttaatgaggcgcgcccgcattccgatttaccgtcaaaagctgcggcgatggtacgtgaaaacgtcattgctcagttggctaatttgcaaactcatccatcggtgcgcctggcgctcgaagaggggcggatcgccctgcacggctgggtctacgacattgaaagcggcagcatcgcagcttttgacggcgcaacccgccagtttgtgccactggccgctaatcctcgcgtttgtgccataccgctacgccaaccgaccgcagcgtaa

SEQ ID NO: 4 - protein, 384 aa, Escherichia coli
MLLVLVLIGLNMRPLLTSVGPLLPQLRQASGMSFSVAALLTALPVVTMGGLALAGSWLHQHVSERRSVAISLLLIAVGALMRELYPQSALLLSSALLGGVGIGIIQAVMPSVIKRRFQQRTPLVMGLWSAALMGGGGLGAAITPWLVQHSETWYQTLAWWALPAVVALFAWWWQSAREVASSHKTTTTPVRVVFTPRAWTLGVYFGLINGGYASLIAWLPAFYIEIGASAQYSGSLLALMTLGQAAGALLMPAMARHQDRRKLLMLALVLQLVGFCGFIWLPMQLPVLWAMVCGLGLGGAFPLCLLLALDHSVQPAIAGKLVAFMQGIGFIIAGLAPWFSGVLRSISGNYLMDWAFHALCVVGLMIITLRFAPVRFPQLWVKEA

SEQ ID NO: 5 - protein, 219 aa, Escherichia coli
MKEIIDGFLKFQREAFPKREALFKQLATQQSPRTLFISCSDSRLVPELVTQREPGDLFVIRNAGNIVPSYGPEPGGVSASVEYAVAALRVSDIVICGHSNCGAMTAIASCQCMDHMPAVSHWLRYADSARVVNEARPHSDLPSKAAAMVRENVIAQLANLQTHPSVRLALEEGRIALHGWVYDIESGSIAAFDGATRQFVPLAANPRVCAIPLRQPTAA

SEQ ID NO: 6 - protein, 293 aa, Escherichia coli
MILGTALTGLFSVVAQILVPLAATLASPDKRGKVVGTIMSGLLLGILLARTVAGLLANLGGWRTVFWVASVLMALMALALWRGLPQMKSETHLNYPQLLGSVFSMFISDKILRTRALLGCLTFANFSILWTSMAFLLAAPPFNYSDGVIGLFGLAGAAGALGARPAGGFADKGKSHHTTTFGLLLLLLSWLAIWFGHTSVLALIIGILVLDLTVQGVHITNQTVIYRIHPDARNRLTAGYMTSYFIGGAAGSLISASAWQHGGWAGVCLAGATIALVNLLVWWRGFHRQEAAN

SEQ ID NO: 7 - DNA, 882 bp, Escherichia coli
  source 1..882: mol_type = genomic DNA
atgatcctcggtacggcattaaccggtttattctcagtcgtggcacaaattctggttccgctggcagcgacgctggcttcaccggataaacgcggcaaagtggttggcactattatgagcggtctgctgttggggatcttgctggcacggacagttgccggattgctggcgaatctcggcggctggcgcaccgtcttttgggttgcttcggtgttaatggcactgatggcgctggcattatggcgtggtctgccacaaatgaaatcagaaacccacctcaactacccacagttgttgggttccgttttcagtatgtttatcagcgataaaattctgcgtacccgcgcgttgctgggctgcctgacctttgccaatttcagcattctctggacctcaatggcctttttgcttgccgctccaccttttaactacagcgatggtgtcattggtctgtttggacttgcgggagctgccggagcgttgggcgctcgtccggcgggcggttttgccgataagggcaaatcgcaccacaccacaactttcggtctgctgctgctattactttcatggctggcgatctggtttggtcacacttccgtactggcgttgattatcggaatcctggtgctggatctcaccgtgcagggcgtgcatatcactaaccagacggtaatttatcggatacatcctgatgcgcgcaatcgcctgaccgcaggttacatgactagctactttattggcggtgccgccggttcgctaatttcagcctcagcctggcaacatggcggttgggctggcgtttgtctggctggcgcgacgattgccctggttaacttactggtctggtggcgaggttttcatcgtcaggaagccgcaaattaa

SEQ ID NO: 8 - DNA, 2462 bp, synthetic construct
  source 1..2462: mol_type = other DNA
cctacaaaccacatcgcacatttcaacaatctatctttcatcccatattcatcaacatccgctattattgatttccagcttaatcatcacctgatgaacaaaaataatgactaaacctaatcatgagcttagcccggcgctgatcgtgctgatgtctatcgccaccggtctggcggtagccagtaactattacgcccagccattgctcgacaccatcgcgcgtaacttttccctttccgccagttcggcaggctttattgttaccgccgcgcagttgggctatgccgcaggtctactgtttcttgttcccctcggtgatatgtttgaacgccgccgcctgattgtctcgatgaccttactggcggcatgttgattaccgccagcagtcagtcgctggcgatgatgatcctcggtacggcattaaccggtttattctcagtcgtggcacaaattctggttccgctggcagcgacgctggcttcaccggataaacgcggcaaagtggttggcactattatgagcggtctgctgttggggatcttgctggcacggacagttgccggattgctggcgaatctcggcggctggcgcaccgtcttttgggttgcttcggtgtttgacaattaatcatccggctcgtataatgtgtggaattgtgagcggataacaatttcacacaggaaacagaccatgctgctggtactggtgctgattggtcttaatatgcgaccactgctcacctccgtcgggccactgctaccgcaattgcgccaggcgagcggaatgagctttagcgtggctgccctgttgaccgctctgccggtggttaccatgggcgggctggcgctggccggaagctggcttcatcagcatgtcagcgaacgtcgcagtgtcgccatcagtctgttgctgattgccgtcggtgcattgatgcgtgagctttacccgcaaagtgcgctgctgcttagcagcgcactgcttggtggggtggggatcggcatcattcaggcggtgatgccttcggtgattaaacggcggtttcagcagcgcacgccactggtgatggggctgtggtccgcggctctgatgggcggcggtgggcttggtgccgccataacgccctggttagttcaacatagcgaaacctggtatcaaacactcgcctggtgggcgctgcctgccgttgttgcgctctttgcctggtggtggcaaagcgcccgcgaggtcgcctcttcccacaagacaacaaccactccggttcgcgtggtattcactccccgcgcgtggacgctgggtgtttacttcggtctgattaacggcggttacgccagcctgattgcctggttacccgctttctatattgagattggtgccagcgcgcagtacagcggttccttactggcattgatgacgcttgggcaagccgcaggagctttgctgatgcctgctatggctcgccatcaggatcggcgcaaactgttaatgctggcgctggtgttacaactggtggggttctgcggctttatctggctgccgatgcaattgccggtattgtgggcgatggtgtgtgggttaggtctgggcggcgcgtttccgctctgtttgctgctggcgctcgatcactctgtgcaaccggctattgctggcaagctggtggcgtttatgcagggaatcggttttatcatcgccgggcttgccccgtggttttctggcgtgctgcgtagtatcagcggcaattacctgatggactgggcatttcatgcgctgtgcgtcgttgggctgatgatcataaccctgcgttttgcaccagtacgttttccgcagctgtgggtcaaagaggcatgattgcttgccgctccaccttttaactacagcgatggtgtcattggtctgtttggacttgcgggagctgccggagcgttgggcgctcgtccggcgggcggttttgccgataagggcaaatcgcaccacaccacaactttcggtctgctgctgctattactttcatggctggcgatctggtttggtcacacttccgtactggcgttgattatcggaatcctggtgctggatctcaccgtgcagggcgtgcatatcactaaccagacggtaatttatcggatacatcctgatgcgcgcaatcgcctgaccgcaggttacatgactagctactttattggcggtgccgccggttcgctaatttcagcctcagcctggcaacatggcggttgggctggcgtttgtctggctggcgcgacgattgccctggttaacttactggtctggtggcgaggttttcatcgtcaggaagccgcaaattaagcaatcagcaaccgttttcgtggctttacacttataagggtgttaagaagcccatcagtctgataaggttaagatattcattcagtctatttataatattaacaatcgttaagcgtacactctatggaaagccctactcc

SEQ ID NO: 9 - DNA, 1099 bp, synthetic construct
  source 1..1099: mol_type = other DNA
gtttgtgccataccgctacgccaaccgaccgcagcgtaaccttatttttaaaccatcaggagttccaccatgattcagtcacaaattaaccgcaatattcgtcttgatcttgccgatgccattttgctcagcaaagctaaaaaagatctctcatttgccgagattgccgacggcaccggtctggcagaagcctttgtaaccgcggctttgctgggtcagcaggcgcttcctgccgacgccgcccgcctggtcggggcgaagctggatctcgacgaagactccattctactgttgcagatgattccactgcgtggctgcattgatgaccgtattccaactgacccaacgatgtatcgtttctatgaaatgttgcaggtgtacggtacaaccctgaaagcgttggttcatgagaaatttggcgatggcattattagcgcgattaacttcaaactcgacgttaagaaagtggcggacccggaaggtggcgaacgtgcggtcatcaccttagatggtaaatatctgccgaccaaaccgttctgacagccatgcgcaaccatcaaaagacgttcacgtgcgacgcttgttcctgcgctttgttcatgccggatgcggctaatgtagatcgctgaacttgtaggcctgataagcgcagcgtatcaggcaatttttataatttaaactgacgattcaactttataatctttgaaataatagtgcttatcccggtcgtttatttcgcgaataacccgacaaggaacgccagccgccacgacgtttggtggaatgtcttttgtgacgatactacccgcgccaataacagaattatccccgatggtgacgcctggattaataaccacatgacttccgatccagacgttattgccaatcgttatcggaaaagagtacatctcgccgttttttctcaattcatggtgtacagggtgtcccgtaacggaaagagtaacgttgggtgcaatcagtacgttatcaccgattgttaccgtgtagtcatcgacaatggttaaattgaaatttgcataaaaattgcggcctatatggatgttggaaccgtaagagaaatagacaggcggttctaccc

SEQ ID NO: 10 - DNA, 1967 bp, synthetic construct
  source 1..1967: mol_type = other DNA
cctacaaaccacatcgcacatttcaacaatctatctttcatcccatattcatcaacatccgctattattgatttccagcttaatcatcacctgatgaacaaaaataatgactaaacctaatcatgagcttagcccggcgctgatcgtgctgatgtctatcgccaccggtctggcggtagccagtaactattacgcccagccattgctcgacaccatcgcgcgtaacttttccctttccgccagttcggcaggctttattgttaccgccgcgcagttgggctatgccgcaggtctactgtttcttgttcccctcggtgatatgtttgaacgccgccgcctgattgtctcgatgaccttactggcggcatgttgattaccgccagcagtcagtcgctggcgatgatgatcctcggtacggcattaaccggtttattctcagtcgtggcacaaattctggttccgctggcagcgacgctggcttcaccggataaacgcggcaaagtggttggcactattatgagcggtctgctgttggggatcttgctggcacggacagttgccggattgctggcgaatctcggcggctggcgcaccgtcttttgggttgcttcggtgtttgacaattaatcatccggctcgtataatgtgtggaattgtgagcggataacaatttcacacaggaaacagaccgtgaaagagattattgatggattccttaaattccagcgcgaggcatttccgaagcgggaagccttgtttaaacagctggcgacacagcaaagcccgcgcacactttttatctcctgctccgacagccgtctggtccctgagctggtgacgcaacgtgagcctggcgatctgttcgttattcgcaacgcgggcaatatcgtcccttcctacgggccggaacccggtggcgtttctgcttcggtggagtatgccgtcgctgcgcttcgggtatctgacattgtgatttgtggtcattccaactgtggcgcgatgaccgccattgccagctgtcagtgcatggaccatatgcctgccgtctcccactggctgcgttatgccgattcagcccgcgtcgttaatgaggcgcgcccgcattccgatttaccgtcaaaagctgcggcgatggtacgtgaaaacgtcattgctcagttggctaatttgcaaactcatccatcggtgcgcctggcgctcgaagaggggcggatcgccctgcacggctgggtctacgacattgaaagcggcagcatcgcagcttttgacggcgcaacccgccagtttgtgccactggccgctaatcctcgcgtttgtgccataccgctacgccaaccgaccgcagcgtaattgcttgccgctccaccttttaactacagcgatggtgtcattggtctgtttggacttgcgggagctgccggagcgttgggcgctcgtccggcgggcggttttgccgataagggcaaatcgcaccacaccacaactttcggtctgctgctgctattactttcatggctggcgatctggtttggtcacacttccgtactggcgttgattatcggaatcctggtgctggatctcaccgtgcagggcgtgcatatcactaaccagacggtaatttatcggatacatcctgatgcgcgcaatcgcctgaccgcaggttacatgactagctactttattggcggtgccgccggttcgctaatttcagcctcagcctggcaacatggcggttgggctggcgtttgtctggctggcgcgacgattgccctggttaacttactggtctggtggcgaggttttcatcgtcaggaagccgcaaattaagcaatcagcaaccgttttcgtggctttacacttataagggtgttaagaagcccatcagtctgataaggttaagatattcattcagtctatttataatattaacaatcgttaagcgtacactctatggaaagccctactcc

SEQ ID NO: 11 - DNA, 1062 bp, synthetic construct
  source 1..1062: mol_type = other DNA
aatcccaacgtccaactcgtcgcggcaaagcatatcctcgattttctcctgcgacatttcctgtagctggagcgtgatgctgggatagcgcgcatagaaatccgccattaaggggccgataaagtagctcgtaaaggtgggggtgacggcgatacgcagcgatcctcgcgtcagatcggcaacatcatgaatcgcccgtttacccgcccccagttcctgtaacgcccggctggcgtactgtcgccagacttctcctgcatcagtgagacgaatcgttcgcccgctacggtcaaacagcggcacgcctaaactctcctctaactggcgaatctgctgggaaagcgcaggttgggagacgtgcaacgcactggcggcacgggtgaagctgccatgttcagccacggcaagaaaataattgatatgtcgagagagcattcgcaacctataagtaaatccaatggaactcatcataaatgagacttttaccttatgacaatcggcgagtagtctgcctctcattccagagacagacagaggttaacgccttatttttaaaccatcaggagttccaccatgattcagtcacaaattaaccgcaatattcgtcttgatcttgccgatgccattttgctcagcaaagctaaaaaagatctctcatttgccgagattgccgacggcaccggtctggcagaagcctttgtaaccgcggctttgctgggtcagcaggcgcttcctgccgacgccgcccgcctggtcggggcgaagctggatctcgacgaagactccattctactgttgcagatgattccactgcgtggctgcattgatgaccgtattccaactgacccaacgatgtatcgtttctatgaaatgttgcaggtgtacggtacaaccctgaaagcgttggttcatgagaaatttggcgatggcattattagcgcgattaacttcaaactcgacgttaagaaagtggcggacccggaaggtggcgaacgtgcggtcatcaccttagatggtaaatatctgccgaccaaaccgttctgacagccatgcgcaaccatc

SEQ ID NO: 12 - DNA, 22 bp, synthetic construct
  source 1..22: mol_type = other DNA
cctacaaaccacatcgcacatt

SEQ ID NO: 13 - DNA, 76 bp, synthetic construct
  source 1..76: mol_type = other DNA
aattgttatccgctcacaattccacacattatacgagccggatgattaattgtcaaacaccgaagcaacccaaaag

SEQ ID NO: 14 - DNA, 85 bp, synthetic construct
  source 1..85: mol_type = other DNA
tccggctcgtataatgtgtggaattgtgagcggataacaatttcacacaggaaacagaccgtgaaagagattattgatggattcc

SEQ ID NO: 15 - DNA, 36 bp, synthetic construct
  source 1..36: mol_type = other DNA
ggtggagcggcaagcaattacgctgcggtcggttgg

SEQ ID NO: 16 - DNA, 36 bp, synthetic construct
  source 1..36: mol_type = other DNA
ccaaccgaccgcagcgtaattgcttgccgctccacc

SEQ ID NO: 17 - DNA, 24 bp, synthetic construct
  source 1..24: mol_type = other DNA
ggagtagggctttccatagagtgt

SEQ ID NO: 18 - DNA, 56 bp, synthetic construct
  source 1..56: mol_type = other DNA
agtcctaggtataatactagtctcaactacccacagttgttgttttagagctagaa

SEQ ID NO: 19 - DNA, 56 bp, synthetic construct
  source 1..56: mol_type = other DNA
ttctagctctaaaacaacaactgtgggtagttgagactagtattatacctaggact

SEQ ID NO: 20 - DNA, 61 bp, synthetic construct
  source 1..61: mol_type = other DNA
tgagcggataacaatttcacacaggaaacagaattcgtgaaagagattattgatggattcc

SEQ ID NO: 21 - DNA, 55 bp, synthetic construct
  source 1..55: mol_type = other DNA
tctcatccgccaaaacagaagcttggctgcaggtcgacttacgctgcggtcggtt

SEQ ID NO: 22 - DNA, 23 bp, synthetic construct
  source 1..23: mol_type = other DNA
agcggataacaatttcacacagg

SEQ ID NO: 23 - DNA, 20 bp, synthetic construct
  source 1..20: mol_type = other DNA
caggctgaaaatcttctctc

SEQ ID NO: 24 - DNA, 19 bp, synthetic construct
  source 1..19: mol_type = other DNA
aatcccaacgtccaactcg

SEQ ID NO: 25 - DNA, 44 bp, synthetic construct
  source 1..44: mol_type = other DNA
actcctgatggtttaaaaataaggcgttaacctctgtctgtctc

SEQ ID NO: 26 - DNA, 44 bp, synthetic construct
  source 1..44: mol_type = other DNA
gagacagacagaggttaacgccttatttttaaaccatcaggagt

SEQ ID NO: 27 - DNA, 18 bp, synthetic construct
  source 1..18: mol_type = other DNA
gatggttgcgcatggctg

SEQ ID NO: 28 - DNA, 56 bp, synthetic construct
  source 1..56: mol_type = other DNA
agtcctaggtataatactagtatttgtggtcattccaactggttttagagctagaa

SEQ ID NO: 29 - DNA, 56 bp, synthetic construct
  source 1..56: mol_type = other DNA
ttctagctctaaaaccagttggaatgaccacaaatactagtattatacctaggact

SEQ ID NO: 30 - DNA, 24 bp, synthetic construct
  source 1..24: mol_type = other DNA
ctagtattatacctaggactgagc

SEQ ID NO: 31 - DNA, 24 bp, synthetic construct
  source 1..24: mol_type = other DNA
gttttagagctagaaatagcaagt

SEQ ID NO: 32 - DNA, 20 bp, synthetic construct
  source 1..20: mol_type = other DNA
gcagtggcggttttcatggc

SEQ ID NO: 33 - DNA, 23 bp, synthetic construct
  source 1..23: mol_type = other DNA
ccttggtgatctcgcctttcacg

SEQ ID NO: 34 - DNA, 80 bp, synthetic construct
  source 1..80: mol_type = other DNA
tccggctcgtataatgtgtggaattgtgagcggataacaatttcacacaggaaacagaccatgctgctggtactggtgct

SEQ ID NO: 35 - DNA, 36 bp, synthetic construct
  source 1..36: mol_type = other DNA
ggtggagcggcaagcaatcatgcctctttgacccac

SEQ ID NO: 36 - DNA, 36 bp, synthetic construct
  source 1..36: mol_type = other DNA
gtgggtcaaagaggcatgattgcttgccgctccacc

SEQ ID NO: 37 - DNA, 24 bp, synthetic construct
  source 1..24: mol_type = other DNA
ggagtagggctttccatagagtgt

SEQ ID NO: 38 - DNA, 54 bp, synthetic construct
  source 1..54: mol_type = other DNA
tgagcggataacaatttcacacaggaaacagaattcatgctgctggtactggtg

SEQ ID NO: 39 - DNA, 57 bp, synthetic construct
  source 1..57: mol_type = other DNA
tctcatccgccaaaacagaagcttggctgcaggtcgactcatgcctctttgacccac

SEQ ID NO: 40 - DNA, 20 bp, synthetic construct
  source 1..20: mol_type = other DNA
gtttgtgccataccgctacg

SEQ ID NO: 41 - DNA, 38 bp, synthetic construct
  source 1..38: mol_type = other DNA
cgcaggaacaagcgtcgcacgtgaacgtcttttgatgg

SEQ ID NO: 42 - DNA, 38 bp, synthetic construct
  source 1..38: mol_type = other DNA
ccatcaaaagacgttcacgtgcgacgcttgttcctgcg

SEQ ID NO: 43 - DNA, 20 bp, synthetic construct
  source 1..20: mol_type = other DNA
gggtagaaccgcctgtctat

SEQ ID NO: 44 - DNA, 56 bp, synthetic construct
  source 1..56: mol_type = other DNA
agtcctaggtataatactagtactgctaccgcaattgcgccgttttagagctagaa

SEQ ID NO: 45 - DNA, 56 bp, synthetic construct
  source 1..56: mol_type = other DNA
ttctagctctaaaacggcgcaattgcggtagcagtactagtattatacctaggact

SEQ ID NO: 46 - DNA, 20 bp, synthetic construct
  source 1..20: mol_type = other DNA
ctcaactacccacagttgtt

SEQ ID NO: 47 - DNA, 20 bp, synthetic construct
  source 1..20: mol_type = other DNA
atttgtggtcattccaactg

SEQ ID NO: 48 - DNA, 20 bp, synthetic construct
  source 1..20: mol_type = other DNA
actgctaccgcaattgcgcc

SEQ ID NO: 49 - DNA, 25 bp, synthetic construct
  source 1..25: mol_type = other DNA
gctcagtcctaggtataatactagt

SEQ ID NO: 50 - DNA, 36 bp, synthetic construct
  source 1..36: mol_type = other DNA
tgagcggataacaatttcacacaggaaacagaattc

SEQ ID NO: 51 - DNA, 38 bp, synthetic construct
  source 1..38: mol_type = other DNA
tctcatccgccaaaacagaagcttggctgcaggtcgac